European Patent Application EP 4 201 951 A1, published June 28, 2023. Title: Method for peptide synthesis. Applicant: Bachem Holding AG. The sequence listing filed with the application follows.

SEQUENCE LISTING (8 sequences)

SEQ ID NO: 1 - protein, 4 aa, Artificial Sequence
  synthesized peptide
HPFA

SEQ ID NO: 2 - protein, 5 aa, Artificial Sequence
  synthesized peptide
HHPFA

SEQ ID NO: 3 - protein, 4 aa, Artificial Sequence
  synthesized peptide
  Xaa (2)..(2): N-methylalanine
CXFA

SEQ ID NO: 4 - protein, 5 aa, Artificial Sequence
  synthesized peptide
  Xaa (3)..(3): N-methylalanine
CCXFA

SEQ ID NO: 5 - protein, 4 aa, Artificial Sequence
  synthesized peptide
  Xaa (1)..(1): alpha-phenylglycine
  Xaa (2)..(2): N-methylalanine
XXFA

SEQ ID NO: 6 - protein, 5 aa, Artificial Sequence
  synthesized peptide
  Xaa (1)..(1): alpha-phenylglycine
  Xaa (2)..(2): alpha-phenylglycine
  Xaa (3)..(3): N-methylalanine
XXXFA

SEQ ID NO: 7 - protein, 4 aa, Artificial Sequence
  synthesized peptide
  Xaa (2)..(2): alpha-aminoisobutyric acid
  Ala (4)..(4): AMIDATION
HXFA

SEQ ID NO: 8 - protein, 5 aa, Artificial Sequence
  synthesized peptide
  Xaa (3)..(3): alpha-aminoisobutyric acid
  Ala (5)..(5): AMIDATION
HHXFA